European Patent Specification EP 3 997 212 B1, published March 18, 2026. Title: ENGINEERED REGULATORY T CELLS. Applicant: THE CHILDREN'S MERCY HOSPITAL THE UNIVERSITY OF KANSAS. The sequence listing filed with the application follows.

SEQUENCE LISTING (12 sequences)

SEQ ID NO: 1 - DNA, 1578 bp, Artificial Sequence
  IKZF2 cDNA encoding full length Helios
atggaaacagaggctattgatggctatataacgtgtgacaatgagctttcacccgaaagggagcactccaatatggcaattgacctcacctcaagcacacccaatggacagcatgcctcaccaagtcacatgacaagcacaaattcagtaaagctagaaatgcagagtgatgaagagtgtgacaggaaacccctgagccgtgaagatgagatcaggggccatgatgagggtagcagcctagaagaacccctaattgagagcagcgaggtggctgacaacaggaaagtccaggagcttcaaggcgagggaggaatccggcttccgaatggtaaactgaaatgtgacgtctgtggcatggtttgcattgggcccaatgtgcttatggtacataaaaggagtcacactggtgaacgccccttccactgtaaccagtgtggagcttcttttactcagaagggcaaccttctgagacacataaagttacactctggagagaagccgttcaaatgtcctttctgtagctacgcctgtagaagaagggacgccctcacaggacacctcaggacccattctgtgggtaaacctcacaagtgcaactactgtggacgaagctacaagcagcgcagttcactggaggagcacaaggaacgctgccacaactatctccagaatgtcagcatggaggctgctgggcaggtcatgagtcaccatgtacctcctatggaagattgtaaggaacaagagcctattatggacaacaatatttctctggtgccttttgagagacctgctgtcatagagaagctcacggggaatatgggaaaacgtaaaagctccactccacaaaagtttgtgggggaaaagctcatgcgattcagctacccagatattcactttgatatgaacttaacatatgagaaggaggctgagctgatgcagtctcatatgatggaccaagccatcaacaatgcaatcacctaccttggagctgaggcccttcaccctctgatgcagcacccgccaagcacaatcgctgaagtggccccagttataagctcagcttattctcaggtctatcatccaaataggatagaaagacccattagcagggaaactgctgatagtcatgaaaacaacatggatggccccatctctctcatcagaccaaagagtcgaccccaggaaagagaggcctctcccagcaatagctgcctggattccactgactcagaaagcagccatgatgaccaccagtcctaccaaggacaccctgccttaaatcccaagaggaaacaaagcccagcttacatgaaggaggatgtcaaagctttggatactaccaaggctcctaagggctctctgaaggacatctacaaggtcttcaatggagaaggagaacagattagggccttcaagtgtgagcactgccgagtccttttcctagaccatgtcatgtacaccattcacatgggttgccatggctaccgggacccactggaatgcaacatctgtggctacagaagccaggaccgttatgagttttcatcacacattgttcgaggggagcacacattccac

SEQ ID NO: 2 - protein, 526 aa, Homo sapiens [sequence omitted]

SEQ ID NO: 3 - DNA, 1287 bp, Artificial Sequence
  FOXP3 codon optimized cDNA
aaccccagacccggaaagccttctgccccttctctggccctgggaccttctcctggcgcctccccatcttggagagccgcccctaaagccagcgatctgctgggagctagaggccctggcggcacatttcagggcagggatctgagaggcggagcccacgcttctagcagcagcctgaaccccatgccccctagccagctgcagctgcctacactgcctctcgtgatggtggcccctagcggagctagactgggccctctgcctcatctgcaggccctgctgcaggacagaccccacttcatgcaccagctgagcaccgtggatgcccacgccagaacacctgtgctgcaggtgcaccccctggaaagccctgccatgatcagcctgaccccccctacaaccgctaccggcgtgttcagcctgaaggccagacctggactgccccctggcatcaatgtggccagcctggaatgggtgtcccgcgaacctgccctgctgtgcaccttccccaatcccagcgcccccagaaaggacagcacactgtctgccgtgccccagagcagctatcccctgctggctaacggcgtgtgcaagtggcctggctgcgagaaggtgttcgaggaacccgaggacttcctgaagcactgccaggccgaccatctgctggacgagaaaggcagagcccagtgtctgctgcagcgcgagatggtgcagagcctggaacagcagctggtgctggaaaaagaaaagctgagcgccatgcaggcccacctggctggaaagatggccctgacaaaggccagcagcgtggccagctctgacaagggcagctgctgcattgtggccgctggctctcagggacctgtggtgcctgcttggagcggacctagagaggcccccgatagcctgtttgccgtgcggagacacctgtggggcagccacggcaactctaccttccccgagttcctgcacaacatggactacttcaagttccacaacatgaggccccccttcacctacgccaccctgatcagatgggccattctggaagcccccgagaagcagcggaccctgaacgaaatctaccactggtttacccggatgttcgccttcttcagaaaccaccccgccacctggaagaacgccatccggcacaatctgagcctgcacaagtgcttcgtgcgggtggaaagcgagaagggcgccgtgtggacagtggacgagctggaatttcggaagaagcggtcccagaggcccagccggtgtagcaatcctacacctggacct

SEQ ID NO: 4 - protein, 429 aa, Artificial Sequence
  FOXP3 codon optimized protein sequence
NPRPGKPSAPSLALGPSPGASPSWRAAPKASDLLGARGPGGTFQGRDLRGGAHASSSSLNPMPPSQLQLPTLPLVMVAPSGARLGPLPHLQALLQDRPHFMHQLSTVDAHARTPVLQVHPLESPAMISLTPPTTATGVFSLKARPGLPPGINVASLEWVSREPALLCTFPNPSAPRKDSTLSAVPQSSYPLLANGVCKWPGCEKVFEEPEDFLKHCQADHLLDEKGRAQCLLQREMVQSLEQQLVLEKEKLSAMQAHLAGKMALTKASSVASSDKGSCCIVAAGSQGPVVPAWSGPREAPDSLFAVRRHLWGSHGNSTFPEFLHNMDYFKFHNMRPPFTYATLIRWAILEAPEKQRTLNEIYHWFTRMFAFFRNHPATWKNAIRHNLSLHKCFVRVESEKGAVWTVDELEFRKKRSQRPSRCSNPTPGP

SEQ ID NO: 5 - DNA, 1500 bp, Artificial Sequence
  IKZF2 cDNA encoding shortened Helios isoform
atggaaacagaggctattgatggctatataacgtgtgacaatgagctttcacccgaaagggagcactccaatatggcaattgacctcacctcaagcacacccaatggacagcatgcctcaccaagtcacatgacaagcacaaattcagtaaagctagaaatgcagagtgatgaagagtgtgacaggaaacccctgagccgtgaagatgagatcaggggccatgatgagggtagcagcctagaagaacccctaattgagagcagcgaggtggctgacaacaggaaagtccaggagcttcaaggcgagggaggaatccggcttccgaatggtgaacgccccttccactgtaaccagtgtggagcttcttttactcagaagggcaaccttctgagacacataaagttacactctggagagaagccgttcaaatgtcctttctgtagctacgcctgtagaagaagggacgccctcacaggacacctcaggacccattctgtgggtaaacctcacaagtgcaactactgtggacgaagctacaagcagcgcagttcactggaggagcacaaggaacgctgccacaactatctccagaatgtcagcatggaggctgctgggcaggtcatgagtcaccatgtacctcctatggaagattgtaaggaacaagagcctattatggacaacaatatttctctggtgccttttgagagacctgctgtcatagagaagctcacggggaatatgggaaaacgtaaaagctccactccacaaaagtttgtgggggaaaagctcatgcgattcagctacccagatattcactttgatatgaacttaacatatgagaaggaggctgagctgatgcagtctcatatgatggaccaagccatcaacaatgcaatcacctaccttggagctgaggcccttcaccctctgatgcagcacccgccaagcacaatcgctgaagtggccccagttataagctcagcttattctcaggtctatcatccaaataggatagaaagacccattagcagggaaactgctgatagtcatgaaaacaacatggatggccccatctctctcatcagaccaaagagtcgaccccaggaaagagaggcctctcccagcaatagctgcctggattccactgactcagaaagcagccatgatgaccaccagtcctaccaaggacaccctgccttaaatcccaagaggaaacaaagcccagcttacatgaaggaggatgtcaaagctttggatactaccaaggctcctaagggctctctgaaggacatctacaaggtcttcaatggagaaggagaacagattagggccttcaagtgtgagcactgccgagtccttttcctagaccatgtcatgtacaccattcacatgggttgccatggctaccgggacccactggaatgcaacatctgtggctacagaagccaggaccgttatgagttttcatcacacattgttcgaggggagcacacattccac

SEQ ID NO: 6 - protein, 500 aa, Homo sapiens
  MISC_FEATURE (1)..(500): Helios shortened isoform
METEAIDGYITCDNELSPEREHSNMAIDLTSSTPNGQHASPSHMTSTNSVKLEMQSDEECDRKPLSREDEIRGHDEGSSLEEPLIESSEVADNRKVQELQGEGGIRLPNGERPFHCNQCGASFTQKGNLLRHIKLHSGEKPFKCPFCSYACRRRDALTGHLRTHSVGKPHKCNYCGRSYKQRSSLEEHKERCHNYLQNVSMEAAGQVMSHHVPPMEDCKEQEPIMDNNISLVPFERPAVIEKLTGNMGKRKSSTPQKFVGEKLMRFSYPDIHFDMNLTYEKEAELMQSHMMDQAINNAITYLGAEALHPLMQHPPSTIAEVAPVISSAYSQVYHPNRIERPISRETADSHENNMDGPISLIRPKSRPQEREASPSNSCLDSTDSESSHDDHQSYQGHPALNPKRKQSPAYMKEDVKALDTTKAPKGSLKDIYKVFNGEGEQIRAFKCEHCRVLFLDHVMYTIHMGCHGYRDPLECNICGYRSQDRYEFSSHIVRGEHTFH

SEQ ID NO: 7 - DNA, 24 bp, Artificial Sequence
  Forward primer
tgatggctatataacgtgtgacaa

SEQ ID NO: 8 - DNA, 22 bp, Artificial Sequence
  Reverse primer
ctcacacttgaaggccctaatc

SEQ ID NO: 9 - DNA, 993 bp, Artificial Sequence
  codon optimized delta-CD19
ccccctcggctgctgttcttcctgctgttcctgacccctatggaagtgcggcccgaggaacccctggtcgtgaaagtggaagagggcgacaacgccgtgctgcagtgtctgaagggcacctccgatggccctacccagcagctgacatggtccagagagagccccctgaagcccttcctgaagctgagcctgggactgcctggcctgggcatccatatgaggccactggccatctggctgttcatcttcaacgtgtcccagcagatgggcggcttctacctgtgtcagcctggccccccaagcgagaaagcctggcagcctggctggaccgtgaacgtggaaggatctggcgagctgttccggtggaacgtgtccgatctgggcggactgggctgcggcctgaagaacagaagcagcgagggccctagcagccccagcggcaaactgatgagccccaagctgtacgtgtgggccaaggaccggcccgagatttgggaaggcgagcctccttgcctgccccccagagacagcctgaatcagagcctgagccaggacctgacaatggcccctggcagcacactgtggctgagctgtggcgtgccacccgactctgtgtccagaggccctctgagctggacccacgtgcaccctaagggccctaagagcctgctgtccctggaactgaaggacgacagacccgccagagatatgtgggtcatggaaaccggcctgctgctgcctagagccaccgctcaggatgccggaaagtactactgccaccggggcaacctgaccatgagcttccacctggaaatcaccgccagacccgtgctgtggcactggctgctgagaaccggcggatggaaagtgtccgccgtgaccctggcctacctgatcttctgcctgtgctccctcgtgggcatcctgcatctgcagcgggctctggtgctgcggcggaagagaaagagaatgaccgaccccacccgcagattc

SEQ ID NO: 10 - protein, 331 aa, Artificial Sequence
  truncated delta-CD19
PPRLLFFLLFLTPMEVRPEEPLVVKVEEGDNAVLQCLKGTSDGPTQQLTWSRESPLKPFLKLSLGLPGLGIHMRPLAIWLFIFNVSQQMGGFYLCQPGPPSEKAWQPGWTVNVEGSGELFRWNVSDLGGLGCGLKNRSSEGPSSPSGKLMSPKLYVWAKDRPEIWEGEPPCLPPRDSLNQSLSQDLTMAPGSTLWLSCGVPPDSVSRGPLSWTHVHPKGPKSLLSLELKDDRPARDMWVMETGLLLPRATAQDAGKYYCHRGNLTMSFHLEITARPVLWHWLLRTGGWKVSAVTLAYLIFCLCSLVGILHLQRALVLRRKRKRMTDPTRRF

SEQ ID NO: 11 - DNA, 945 bp, Artificial Sequence
  codon optimized delta-CD34
ctcgttagaagaggcgctagagctggccccagaatgcctagaggatggacagctctgtgcctgctgagcctgctgcctagcggctttatgagcctggacaacaacggcaccgccacacctgaactgcctacacagggcaccttcagcaatgtgtctaccaacgtgtcctaccaagagacaaccacacctagcacactgggcagcacatctctgcaccctgtgtctcagcacggcaatgaggccaccaccaacatcaccgagacaaccgtgaagttcacctctacctccgtgattaccagcgtgtacggcaacaccaacagcagcgtgcagagccagacaagcgtgatcagcaccgtgttcacaacccctgccaatgtgtccacaccagaaaccacactgaagcccagcctgtctcctggaaacgtgtccgatctgagcaccacctctacaagcctggccacctctcctacaaagccctacacaagcagcagccccatcctgagcgatatcaaggccgagatcaagtgcagcggcatccgggaagtgaagctgacccagggcatctgcctggaacagaacaagaccagcagctgcgccgagttcaagaaggacagaggcgaaggactggccagagtgctgtgtggcgaagaacaggccgatgctgatgctggcgctcaagtgtgctctctgctgctggctcagtctgaagtgcggcctcagtgtctgttgctggtgctggccaacagaaccgagatcagcagcaaactgcagctgatgaagaagcaccagagcgacctgaagaagctgggcatcctggacttcaccgagcaggatgtggcctctcaccagagctacagccagaaaaccctgatcgccctggtcacatctggcgctctgctggctgtgctgggaatcaccggctactttctgatgaatcggagattc

SEQ ID NO: 12 - protein, 315 aa, Artificial Sequence
  truncated delta-CD34
LVRRGARAGPRMPRGWTALCLLSLLPSGFMSLDNNGTATPELPTQGTFSNVSTNVSYQETTTPSTLGSTSLHPVSQHGNEATTNITETTVKFTSTSVITSVYGNTNSSVQSQTSVISTVFTTPANVSTPETTLKPSLSPGNVSDLSTTSTSLATSPTKPYTSSSPILSDIKAEIKCSGIREVKLTQGICLEQNKTSSCAEFKKDRGEGLARVLCGEEQADADAGAQVCSLLLAQSEVRPQCLLLVLANRTEISSKLQLMKKHQSDLKKLGILDFTEQDVASHQSYSQKTLIALVTSGALLAVLGITGYFLMNRRF